European Patent Specification EP 3 862 013 B1, published August 7, 2024. Title: Pharmaceutical Composition For Treating Or Preventing Ulcer Or Fistula In Intestinal Tract. Applicant: KURUME UNIVERSITY 3-D Matrix, Ltd. The sequence listing filed with the application follows.

SEQUENCE LISTING (3 sequences)

SEQ ID NO: 1 - protein, 16 aa, Artificial Sequence
  synthetic peptide
RADARADARADARADA

SEQ ID NO: 2 - protein, 13 aa, Artificial Sequence
  synthetic peptide
IEIKIEIKIEIKI

SEQ ID NO: 3 - protein, 13 aa, Artificial Sequence
  synthetic peptide
RLDLRLALRLDLR